European Patent Application EP 4 775 222 A1, published July 15, 2026. Title: Dengue virus vaccine and kit of dengue virus vaccine. Applicant: Kagoshima University. Application JP. The sequence listing filed with the application follows.

SEQUENCE LISTING (11 sequences)

SEQ ID NO: 1 - protein, 900 aa, synthetic construct
GTGNTGETLGEKWKNRLNALGKSEFQIYKKSGIQEVDRTLAKEGIKRGETDHHAVSRGSAKLRWFVERNLVTPEGKVVDLGCGRGGWSYYCGGLKNVKEVKGLTKGGPGHEEPIPMSTYGWNLVRLQSGVDVFFTPPEKCDTLLCDIGESSPNPTVEAGRTLRVLNLVENWLNNNTQFCIKVLNPYMPSVIEKMEALQRKYGGALVRNPLSRNSTHEMYWVSNASGNIVSSVNMISRMLINRFTMRHKKATYEPDVDLGSGTRNIGIESEIPNLDIIGKRIEKIKQEHETSWHYDQDHPYKTWAYHGSYETKQTGSASSMVNGVVRLLTKPWDVIPMVTQMAMTDTTPFGQQRVFKEKVDTRTQEPKEGTKKLMKITAEWLWKELGKKKTPRMCTREEFTRKVRSNAALGAIFTDENKWKSAREAVEDSGFWELVDKERNLHLEGKCETCVYNMMGKREKKLGEFGKAKGSRAIWYMWLGARFLEFEALGFLNEDHWFSRENSLSGVEGEGLHKLGYILRDVSKKEGGAMYADDTAGWDTRITLEDLKNEEMVTNHMEGEHKKLAEAIFKLTYQNKVVRVQRPTPRGTVMDIISRRDQRGSGQVVTYGLNTFTNMEAQLIRQMEGEGIFKSIQHLTVTEEIAVKNWLARVGRERLSRMAISGNDCVVKPLDDRFASALTALNDMGKVRKDIQQWEPSRGWNDWTQVPFCSHHFHELIMKDGRVLVVPCRNQDELIGRARISQGAGWSLRETACLGKSYAQMWSLMYFHRRDLRLAANAICSAVPSHWVPTSRTTWSIHATHEWMTTEDMLTVWNRVWIQENPWMEDKTPVESWEEIPYLGKREDQWCGSLIGLTSRATWAKNIQTAINQVRSLIGNEEYTDYMPSMKRFRREEEEAGVLW

SEQ ID NO: 2 - DNA, 6804 bp, Dengue virus 2
  source 1..6804: mol_type = other DNA
gccttggcgatgggacatgggcagattgacaacttctcactaggagtcttgggaatggcattgttcctggaagaaatgctcaggacccgcgtaggaacgaaacatgcaatattgctagttgcagtttctttcgtgacattgatcacagggaacatgtcttttcgagatttggggagagtgatggttatggtgggcgctactatgacggatgacataggcatgggcgtgacttatcttgccctattagcagccttcaaagtcagaccaacttttgcagctggactactcttgagaaagctgacctccaaggaattaatgatgaccaccataggaatcgtactcctctctcagagcaccataccagagactatacttgaactgactgacgcgctggctttggggatgatggttctcaagatagtgagaaatatggaaaagtatcaactagcagtgactatcatggccatcttgtgcgtcccaaatgcagtgatattacaaaacgcatggaaagtgagctgcacaacactggcagtggtgtccgtttccccattgcttttaacatcctcacagcagaaagcagattggataccactggcgttgacgatcaaaggcctcaatccaacagccattttcttaacaaccctctcaagaactagcaagaaaaggagctggccactaaatgaggctattatggcagtcgggatggtgagcattttagccagttctctcttaaagaatgatattcccatgacaggaccattagtagctggagggcttctcactgtgtgttacgtgctcactggaagatcggctgatttggaactggagagagctgctgacgtaagatgggaagaacaggcagagatatcaggaagtagtccaattctgtcagtaacaatatcggaagatggtagcatgtcgataaaaaatgaagaagaagaacaaacactgaccatactcattaggacaggactgctggtgatatcaggactttttcccgtgtcaataccaatcacggcagctgcatggtacctgtgggaagtgaaaaaacaacgagccggagtattgtgggatgtcccttcacccccacctgtgggaaaggccgaactggaagatggagcctatagaatcaagcagaaagggattctaggatactcgcagatcggagctggagtttacaaagaaggaacattccacacaatgtggcacgtcacacgcggtgctgtcctaatgcataaagggaagagaattgaaccatcatgggcggacgtcaagaaagacctaatatcgtatggaggaggctggaagctagaaggagaatggaaggaaggagaagaagtccaggtcctggcattagagcctggaaagaatccaagagccgtccaaacaaaacccggtctcttcaaaactaacactggaaccataggtgccgtatctctggacttttctcctggaacgtcaggatctccaatcgtcgacaaaaaaggaaaagttgtgggcctttatggcaacggtgtcgtcacaaggagtggaacatatgtgagtgctatagcccagactgaaaaaagcatcgaagacaatccagagattgaagatgacatctttcgaaagaaaagattgaccatcatggacctccacccaggggcgggaaaaacgaagagataccttccagcaatagtcagagaagccataaaacgaggcttgaggacactaattctggcccccactagagttgtggcggctgaaatggaagaagctctcagaggacttccaataagataccaaacccccgccatcagagctgaacacactggacgggagattgtggatctaatgtgtcacgccacatttaccatgaggctgctatccccaattagagtaccaaattacaacctgatcatcatggatgaagcccatttcacagacccagcaagcatagcagctagaggatacatttcaactcgagttgagatgggtgaagcagctgggattttcatgacagctactcctcctggaagcagagacccatttcctcagagcaatgcaccaatcatggatgaagaaagggaaatccctgagcgttcgtggaattctggacatgaatgggttacggattttaaagggaagactgtttggtttgttccaagtataaaagcaggaaatgatatagcagcttgcctgagaaagaatggaaagaaagtgatacaactcagcaggaagacctttgattctgaatatgtcaagactaggaccaatgattgggactttgtggtcacgacagacatttcagaaatgggcgctaacttcaaggctgagagggttatagaccccaggcgctgcatgaaaccagtcatactaacagacggtgaagagcgggtgatcctggcaggacccatgccagtgacccactctagtgcagcacaaagaagaggaagagtaggaagaaatccaaaaaatgaaaatgaccagtacatatacatgggggaacctctggaaaatgatgaagattgtgcacactggaaagaagctaaaatgcttctagataacatcaacacgcctgaaggaatcattcccagtatgttcgaaccagagcgtgaaaaggtggatgccattgatggtgaataccgcttaagaggagaagcgaggaaaacttttgtggacctaatgagaagaggagacctaccagtctggctagcctacagagtggcagctgaaggtatcaactacgcagacagaagatggtgctttgatggagtcaagaacaatcaaatcttggaagaaaatgtggaagtggaaatttggacaaaagaaggagaaaggaagaaattaaaacccagatggttggatgctaggatctactctgacccactggcgctcaaagaattcaaggaattcgcagctggaagaaagtccctgaccctgaatctaatcacagagatgggtaggctcccaaccttcatgacccagaaagcaaggaacgcactagacaacttagcagtcctgcatacggctgaagcaggcggaagggcgtacaatcatgctcttagtgaactgccggagaccttggagacattgcttttactgacactcttggccacagtcacgggcggaatcttcctattcttgatgagcggaaaaggcatagggaagatgaccctgggaatgtgctgcataatcacggccagtgttctcctatggtatgcacaaatacagccacactggatagcagcttcaataatactggagttttttctcatagtcttgctcattccagaaccagaaaagcagagaacaccccaagataaccaattaacttatgttgtcatagccatccttacagtggtggccgcaactatggcaaacgagatgggtttcctggaaaaaacaaagaaagatttcggattgggaagcattgcaacccagcaacctgagagcaacatcctggacatagatctacgtcctgcatcagcttggactctatatgctgtggcaacaactttcatcacaccaatgctgagacacagcattgaaaattcctcagtgaatgtgtctctaacggccattgccaaccaagccacagttttaatgggtcttgggaaaggatggccattgtcaaaaatggacatcggagttccccttctcgctatcgggtgctattcacaagttaaccccataactctcacggcagcccttctcttattggtagcacattatgccatcatagggcctggactccaagcgaaagcaactagagaagctcagaaaagagcagcagcgggcatcatgaaaaacccaactgtggatggaataacagtgattgacctagatccaataccctatgatccaaagtttgaaaagcagttgggacaagtaatgctcttagtcctctgcgtgactcaagtattgatgatgaggactacatgggctttgtgtgaggctctaaccttagcgactgggcccatctccacactgtgggaaggaaatccagggagattttggaatacaactattgcagtatcaatggctaacatttttagagggagctacctggccggagccggacttctcttttctatcatgaagaatacggccaacacaagaaggggaactggcaacacaggagagacgcttggagaaaaatggaaaaaccgattgaatgcattggggaagagtgaattccagatctataagaaaagtggaatccaggaggtggatagaaccttagcaaaagaaggcatcaaaagaggagaaacggaccatcacgctgtgtcgcgaggctcggcgaaactgagatggttcgtcgagagaaacctggtcacaccagaagggaaagtagtggacctcggttgcggcagggggggctggtcatactattgtgggggactaaagaatgtaaaagaagtcaaaggcctaacaaaaggaggaccaggacacgaagaacccattcccatgtcaacatatggttggaacctggtgcgtcttcaaagtggagttgatgttttttttactccgccagaaaagtgtgacacactactgtgtgacataggggagtcgtcaccaaaccccacggtcgaggcaggacgaacactcagagttctaaacctagtggaaaattggctgaacaacaacacccaattttgcatcaaggttctcaacccatatatgccctcagttatagaaaaaatggaagcgctgcaaaggaaatacggaggagctttggtgaggaatccactctcacgaaattccacacacgagatgtactgggtatccaatgcttccgggaacatagtgtcatcagtgaacatgatttcaagaatgttgattaacagattcacaatgagacataagaaggccacatacgagccagatgttgacctcggaagcggaacccgcaacatcggaattgaaagtgagataccaaatttggacataattgggaaaagaatagaaaaaataaaacaagagcatgaaacatcatggcactatgaccaagaccacccatacaaaacgtgggcctaccatggcagctacgaaacaaaacagactggatcggcatcatccatggtgaacggagtggttaggctgctaacaaaaccttgggacgtcatccctatggtgacacagatggcaatgacagacacgactccatttggacaacagcgcgttttcaaagagaaagtggacacgagaacccaagaaccgaaagaaggcacgaaaaaactaatgaaaatcacggcagaatggctctggaaagaactaggaaagaaaaagacacctaggatgtgcaccagagaggaattcacaagaaaggtgagaagcaatgcagccttaggtgccatattcactgatgagaacaagtggaagtcggcacgtgaggctgttgaagatagtggattttgggaactggttgacaaggaaaggaatcttcatcttgaaggaaagtgtgagacatgtgtgtacaacatgatgggaaagagagagaagaagctaggggagttcggcaaagcaaaaggcagcagagccatatggtacatgtggcttggagcacgcttcttagagtttgaagccctaggattcttgaatgaagatcactggttttccagagagaactccctgagtggagtggaaggagaagggctgcacaaactaggctacattttaagagacgtgagcaagaaagaaggaggagcaatgtacgccgatgacaccgcaggatgggacacaaggatcacactggaggacttaaaaaatgaagaaatggtgacaaaccacatggaaggagaacacaagaaacttgctgaagccattttcaaattaacgtaccaaaacaaggtggtgcgtgtgcaaagaccaacaccaagaggcacagtaatggacattatatcaagaagagaccaaagaggtagcggacaagttgtcacctacggcctcaatactttcaccaacatggaagcccaactgatcagacagatggagggagaaggaatcttcaaaagcatccagcacctgacagtcacagaagaaattgcagtgaaaaactggttagcaagagtggggcgtgagaggttatcaagaatggctatcagtggagatgattgtgttgtgaaacccttagatgacaggtttgcaagcgctctaacagctctaaatgacatgggaaaagttaggaaagacatacaacaatgggaaccttcaagaggatggaacgattggacacaagtgcccttttgttcacaccatttccatgagttaatcatgaaggacggtcgtgtactcgtagttccatgcagaaaccaagatgaactgattggtagggcccgaatttcccagggagccgggtggtctttgcgggaaacggcctgtttggggaagtcttacgcccaaatgtggagcctgatgtacttccacagacgtgaccttaggctggcggcaaatgccatttgctcggcagtcccatcacattgggttccaacaagtcgaacaacttggtccatacatgccacacatgagtggatgacaacagaagatatgctgacagtctggaacagggtgtggattcaagaaaacccatggatggaagacaaaactccagtagaatcatgggaggaaatcccatatttggggaaaagagaagaccaatggtgcggctcactgatcgggctaacaagcagggccacctgggcaaagaacatccaaacagcaataaatcaagttagatccctaataggcaatgaggaatacacagactacatgccatccatgaaaaggttcagaagagaagaggaagaggcaggagtcctgtgg

SEQ ID NO: 3 - DNA, 6804 bp, synthetic construct
  misc_feature 1..6804: note = Modified DNA
  source 1..6804: mol_type = other DNA
gccttggcgatgggacatgggcagattgacaacttctcactaggagtcttgggaatggcattgttcctggaagaaatgctcaggacccgcgtaggaacgaaacatgcaatattgctagttgcagtttctttcgtgacattgatcacagggaacatgtcttttcgagatttggggagagtgatggttatggtgggcgctactatgacggatgacataggcatgggcgtgacttatcttgccctattagcagccttcaaagtcagaccaacttttgcagctggactactcttgagaaagctgacctccaaggaattaatgatgaccaccataggaatcgtactcctctctcagagcaccataccagagactatacttgaactgactgacgcgctggctttggggatgatggttctcaagatagtgagaaatatggaaaagtatcaactagcagtgactatcatggccatcttgtgcgtcccaaatgcagtgatattacaaaacgcatggaaagtgagctgcacaacactggcagtggtgtccgtttccccattgcttttaacatcctcacagcagaaagcagattggataccactggcgttgacgatcaaaggcctcaatccaacagccattttcttaacaaccctctcaagaactagcaagaaaaggagctggccactaaatgaggctattatggcagtcgggatggtgagcattttagccagttctctcttaaagaatgatattcccatgacaggaccattagtagctggagggcttctcactgtgtgttacgtgctcactggaagatcggctgatttggaactggagagagctgctgacgtaagatgggaagaacaggcagagatatcaggaagtagtccaattctgtcagtaacaatatcggaagatggtagcatgtcgataaaaaatgaagaagaagaacaaacactgaccatactcattaggacaggactgctggtgatatcaggactttttcccgtgtcaataccaatcacggcagctgcatggtacctgtgggaagtgaaaaaacaacgagccggagtattgtgggatgtcccttcacccccacctgtgggaaaggccgaactggaagatggagcctatagaatcaagcagaaagggattctaggatactcgcagatcggagctggagtttacaaagaaggaacattccacacaatgtggcacgtcacacgcggtgctgtcctaatgcataaagggaagagaattgaaccatcatgggcggacgtcaagaaagacctaatatcgtatggaggaggctggaagctagaaggagaatggaaggaaggagaagaagtccaggtcctggcattagagcctggaaagaatccaagagccgtccaaacaaaacccggtctcttcaaaactaacactggaaccataggtgccgtatctctggacttttctcctggaacgtcaggatctccaatcgtcgacaaaaaaggaaaagttgtgggcctttatggcaacggtgtcgtcacaaggagtggaacatatgtgagtgctatagcccagactgaaaaaagcatcgaagacaatccagagattgaagatgacatctttcgaaagaaaagattgaccatcatggacctccacccaggggcgggaaaaacgaagagataccttccagcaatagtcagagaagccataaaacgaggcttgaggacactaattctggcccccactagagttgtggcggctgaaatggaagaagctctcagaggacttccaataagataccaaacccccgccatcagagctgaacacactggacgggagattgtggatctaatgtgtcacgccacatttaccatgaggctgctatccccaattagagtaccaaattacaacctgatcatcatggatgaagcccatttcacagacccagcaagcatagcagctagaggatacatttcaactcgagttgagatgggtgaagcagctgggattttcatgacagctactcctcctggaagcagagacccatttcctcagagcaatgcaccaatcatggatgaagaaagggaaatccctgagcgttcgtggaattctggacatgaatgggttacggattttaaagggaagactgtttggtttgttccaagtataaaagcaggaaatgatatagcagcttgcctgagaaagaatggaaagaaagtgatacaactcagcaggaagacctttgattctgaatatgtcaagactaggaccaatgattgggactttgtggtcacgacagacatttcagaaatgggcgctaacttcaaggctgagagggttatagaccccaggcgctgcatgaaaccagtcatactaacagacggtgaagagcgggtgatcctggcaggacccatgccagtgacccactctagtgcagcacaaagaagaggaagagtaggaagaaatccaaaaaatgaaaatgaccagtacatatacatgggggaacctctggaaaatgatgaagattgtgcacactggaaagaagctaaaatgcttctagataacatcaacacgcctgaaggaatcattcccagtatgttcgaaccagagcgtgaaaaggtggatgccattgatggtgaataccgcttaagaggagaagcgaggaaaacttttgtggacctaatgagaagaggagacctaccagtctggctagcctacagagtggcagctgaaggtatcaactacgcagacagaagatggtgctttgatggagtcaagaacaatcaaatcttggaagaaaatgtggaagtggaaatttggacaaaagaaggagaaaggaagaaattaaaacccagatggttggatgctaggatctactctgacccactggcgctcaaagaattcaaggaattcgcagctggaagaaagtccctgaccctgaatctaatcacagagatgggtaggctcccaaccttcatgacccagaaagcaaggaacgcactagacaacttagcagtcctgcatacggctgaagcaggcggaagggcgtacaatcatgctcttagtgaactgccggagaccttggagacattgcttttactgacactcttggccacagtcacgggcggaatcttcctattcttgatgagcggaaaaggcatagggaagatgaccctgggaatgtgctgcataatcacggccagtgttctcctatggtatgcacaaatacagccacactggatagcagcttcaataatactggagttttttctcatagtcttgctcattccagaaccagaaaagcagagaacaccccaagataaccaattaacttatgttgtcatagccatccttacagtggtggccgcaactatggcaaacgagatgggtttcctggaaaaaacaaagaaagatttcggattgggaagcattgcaacccagcaacctgagagcaacatcctggacatagatctacgtcctgcatcagcttggactctatatgctgtggcaacaactttcatcacaccaatgctgagacacagcattgaaaattcctcagtgaatgtgtctctaacggccattgccaaccaagccacagttttaatgggtcttgggaaaggatggccattgtcaaaaatggacatcggagttccccttctcgctatcgggtgctattcacaagttaaccccataactctcacggcagcccttctcttattggtagcacattatgccatcatagggcctggactccaagcgaaagcaactagagaagctcagaaaagagcagcagcgggcatcatgaaaaacccaactgtggatggaataacagtgattgacctagatccaataccctatgatccaaagtttgaaaagcagttgggacaagtaatgctcttagtcctctgcgtgactcaagtattgatgatgaggactacatgggctttgtgtgaggctctaaccttagcgactgggcccatctccacactgtgggaaggaaatccagggagattttggaatacaactattgcagtatcaatggctaacatttttagagggagctacctggccggagccggacttctcttttctatcatgaagaatacggccaacacaagaaggggaactggcaacacaggagagacgcttggagaaaaatggaaaaaccgattgaatgcattggggaagagtgaattccagatctataagaaaagtggaatccaggaggtggatagaaccttagcaaaagaaggcatcaaaagaggagaaacggaccatcacgctgtgtcgcgaggctcggcgaaactgagatggttcgtcgagagaaacctggtcacaccagaagggaaagtagtggacctcggttgcggcagggggggctggtcatactattgtgggggactaaagaatgtaaaagaagtcaaaggcctaacaaaaggaggaccaggacacgaagaacccattcccatgtcaacatatggttggaacctggtgcgtcttcaaagtggagttgatgttttttttactccgccagaaaagtgtgacacactactgtgtgacataggggagtcgtcaccaaaccccacggtcgaggcaggacgaacactcagagttctaaacctagtggaaaattggctgaacaacaacacccaattttgcatcaaggttctcaacccatatatgccctcagttatagaaaaaatggaagcgctgcaaaggaaatacggaggagctttggtgaggaatccactctcacgaaattccacacacgagatgtactgggtatccaatgcttccgggaacatagtgtcatcagtgaacatgatttcaagaatgttgattaacagattcacaatgagacataagaaggccacatacgagccagatgttgacctcggaagcggaacccgcaacatcggaattgaaagtgagataccaaatttggacataattgggaaaagaatagaaaaaataaaacaagagcatgaaacatcatggcactatgaccaagaccacccatacaaaacgtgggcctaccatggcagctacgaaacaaaacagactggatcggcatcatccatggtgaacggagtggttaggctgctaacaaaaccttgggacgtcatccctatggtgacacagatggcaatgacagacacgactccatttggacaacagcgcgttttcaaagagaaagtggacacgagaacccaagaaccgaaagaaggcacgaaaaaactaatgaaaatcacggcagaatggctctggaaagaactaggaaagaaaaagacacctaggatgtgcaccagagaggaattcacaagaaaggtgagaagcaatgcagccttaggtgccatattcactgatgagaacaagtggaagtcggcacgtgaggctgttgaagatagtggattttgggaactggttgacaaggaaaggaatcttcatcttgaaggaaagtgtgagacatgtgtgtacaacatgatgggaaagagagagaagaagctaggggagttcggcaaagcaaaaggcagcagagccatatggtacatgtggcttggagcacgcttcttagagtttgaagccctaggattcttgaatgaagatcactggttttccagagagaactccctgagtggagtggaaggagaagggctgcacaaactaggctacattttaagagacgtgagcaagaaagaaggaggagcaatgtacgccgatgacaccgcaggatgggacacaaggatcacactggaggacttaaaaaatgaagaaatggtgacaaaccacatggaaggagaacacaagaaacttgctgaagccattttcaaattaacgtaccaaaacaaggtggtgcgtgtgcaaagaccaacaccaagaggcacagtaatggacattatatcaagaagagaccaaagaggtagcggacaagttgtcacctacggcctcaatactttcaccaacatggaagcccaactgatcagacagatggagggagaaggaatcttcaaaagcatccagcacctgacagtcacagaagaaattgcagtgaaaaactggttagcaagagtggggcgtgagaggttatcaagaatggctatcagtggaaatgattgtgttgtgaaacccttagatgacaggtttgcaagcgctctaacagctctaaatgacatgggaaaagttaggaaagacatacaacaatgggaaccttcaagaggatggaacgattggacacaagtgcccttttgttcacaccatttccatgagttaatcatgaaggacggtcgtgtactcgtagttccatgcagaaaccaagatgaactgattggtagggcccgaatttcccagggagccgggtggtctttgcgggaaacggcctgtttggggaagtcttacgcccaaatgtggagcctgatgtacttccacagacgtgaccttaggctggcggcaaatgccatttgctcggcagtcccatcacattgggttccaacaagtcgaacaacttggtccatacatgccacacatgagtggatgacaacagaagatatgctgacagtctggaacagggtgtggattcaagaaaacccatggatggaagacaaaactccagtagaatcatgggaggaaatcccatatttggggaaaagagaagaccaatggtgcggctcactgatcgggctaacaagcagggccacctgggcaaagaacatccaaacagcaataaatcaagttagatccctaataggcaatgaggaatacacagactacatgccatccatgaaaaggttcagaagagaagaggaagaggcaggagtcctgtgg

SEQ ID NO: 4 - DNA, 118 bp, synthetic construct
  misc_feature 1..118: note = Synthetic DNA
  source 1..118: mol_type = other DNA
gggcggccctgcaggaaaaattgaaaataaatacaaaggttcttgagggttgtgttaaattgaaagcgagaaataatcataaatagccttggcgatgggacatgggcagattgacaac

SEQ ID NO: 5 - DNA, 46 bp, synthetic construct
  misc_feature 1..46: note = Synthetic DNA
  source 1..46: mol_type = other DNA
gggcggcgcgatcgctcacatttaccacaggactcctgcctcttcc

SEQ ID NO: 6 - DNA, 40 bp, synthetic construct
  misc_feature 1..40: note = Synthetic DNA
  source 1..40: mol_type = other DNA
caagaatggctatcagtggaaatgattgtgttgtgaaacc

SEQ ID NO: 7 - DNA, 40 bp, synthetic construct
  misc_feature 1..40: note = Synthetic DNA
  source 1..40: mol_type = other DNA
ggtttcacaacacaatcatttccactgatagccattcttg

SEQ ID NO: 8 - DNA, 593 bp, synthetic construct
  source 1..593: mol_type = other DNA
aagcttaaaaattgaaaataaatacaaaggttcttgagggttgtgttaaattgaaagcgagaaataatcataaatagctttgagtaatgagaatttcgaaaccacatttgagaagtatttccatccagtgctacttgtgtttacttctaaacagtcattttctaactgaagctgaagctggcattcatgtcttcattttgggctgtttcagtgcagggcttcctaaaacagaagccaactgggtgaatgtaataagtgatttgaaaaaaattgaagatcttattcaatctatgcatattgatgctactttatatacggaaagtgatgttcaccccagttgcaaagtaacagcaatgaagtgctttctcttggagttacaagttatttcacttgagtccggagatgcaagtattcatgatacagtagaaaatctgatcatcctagcaaacaacagtttgtcttctaatgggaatgtaacagaatctggatgcaaagaatgtgaggaactggaggaaaaaaatattaaagaatttttgcagagttttgtacatattgtccaaatgttcatcaacacttcttgataatagaagctt

SEQ ID NO: 9 - DNA, 23 bp, synthetic construct
  source 1..23: mol_type = other DNA
acaccacagagttccatcacaga

SEQ ID NO: 10 - DNA, 21 bp, synthetic construct
  source 1..21: mol_type = other DNA
catctcattgaagtcnaggcc

SEQ ID NO: 11 - DNA, 15 bp, synthetic construct
  source 1..15: mol_type = other DNA
cgatggartgctctc